European Patent Specification EP 3 766 896 B1, published November 5, 2025. Title: T CELL RECEPTORS RECOGNIZING HLA-A1- OR HLA-CW7-RESTRICTED MAGE. Applicant: THE UNITED STATES OF AMERICA, AS REPRESENTED BY THE SECRETARY, DEPARTMENT OF HEALTH AND HUMAN SERVICES. Application Not yet assigned. The sequence listing filed with the application follows.

SEQUENCE LISTING (63 sequences)

SEQ ID NO: 1 - protein, 314 aa, Homo sapiens
MPLEQRSQHCKPEEGLEARGEALGLVGAQAPATEEQEAASSSSTLVEVTLGEVPAAESPDPPQSPQGASSLPTTMNYPLWSQSYEDSSNQEEEGPSTFPDLESEFQAALSRKVAELVHFLLLKYRAREPVTKAEMLGSVVGNWQYFFPVIFSKASSSLQLVFGIELMEVDPIGHLYIFATCLGLSYDGLLGDNQIMPKAGLLIIVLAIIAREGDCAPEEKIWEELSVLEVFEGREDSILGDPKKLLTQHFVQENYLEYRQVPGSDPACYEFLWGPRALVETSYVKVLHHMVKISGGPHISYPPLHEWVLREGEE

SEQ ID NO: 2 - protein, 9 aa, Homo sapiens
EVDPIGHLY

SEQ ID NO: 3 - protein, 314 aa, Homo sapiens
MPLEQRSQHCKPEEGLEAQGEALGLVGAQAPATEEQETASSSSTLVEVTLREVPAAESPSPPHSPQGASTLPTTINYTLWSQSDEGSSNEEQEGPSTFPDLETSFQVALSRKMAELVHFLLLKYRAREPFTKAEMLGSVIRNFQDFFPVIFSKASEYLQLVFGIEVVEVVRIGHLYILVTCLGLSYDGLLGDNQIVPKTGLLIIVLAIIAKEGDCAPEEKIWEELSVLEASDGREDSVFAHPRKLLTQDLVQENYLEYRQVPGSDPACYEFLWGPRALVETSYVKVLHHLLKISGGPHISYPPLHEWAFREGEE

SEQ ID NO: 4 - protein, 9 aa, Homo sapiens
VRIGHLYIL

SEQ ID NO: 5 - protein, 6 aa, Homo sapiens
NSASQS

SEQ ID NO: 6 - protein, 6 aa, Homo sapiens
VYSSGN

SEQ ID NO: 7 - protein, 9 aa, Homo sapiens
VVNRDNDMR

SEQ ID NO: 8 - protein, 5 aa, Homo sapiens
KGHDR

SEQ ID NO: 9 - protein, 6 aa, Homo sapiens
SFDVKD

SEQ ID NO: 10 - protein, 12 aa, Homo sapiens
ATSEGGPPYEQY

SEQ ID NO: 11 - protein, 129 aa, Homo sapiens
MISLRVLLVILWLQLSWVWSQRKEVEQDPGPFNVPEGATVAFNCTYSNSASQSFFWYRQDCRKEPKLLMSVYSSGNEDGRFTAQLNRASQYISLLIRDSKLSDSATYLCVVNRDNDMRFGAGTRLTVKP

SEQ ID NO: 12 - protein, 132 aa, Homo sapiens
MASLLFFCGAFYLLGTGSMDADVTQTPRNRITKTGKRIMLECSQTKGHDRMYWYRQDPGLGLRLIYYSFDVKDINKGEISDGYSVSRQAQAKFSLSLESAIPNQTALYFCATSEGGPPYEQYFGPGTRLTVT

SEQ ID NO: 13 - protein, 270 aa, Homo sapiens
MISLRVLLVILWLQLSWVWSQRKEVEQDPGPFNVPEGATVAFNCTYSNSASQSFFWYRQDCRKEPKLLMSVYSSGNEDGRFTAQLNRASQYISLLIRDSKLSDSATYLCVVNRDNDMRFGAGTRLTVKPNIQNPDPAVYQLRDSKSSDKSVCLFTDIDSQTNVSQSKDSDVYITDKTVLDMRSMDFKSNSAVAWSNKSDFACANAFNNSIIPEDTFFPSPESSCDVKLVEKSFETDTNLNFQNLSVIGFRILLLKVAGFNLLMTLRLWSS

SEQ ID NO: 14 - protein, 311 aa, Homo sapiens
MASLLFFCGAFYLLGTGSMDADVTQTPRNRITKTGKRIMLECSQTKGHDRMYWYRQDPGLGLRLIYYSFDVKDINKGEISDGYSVSRQAQAKFSLSLESAIPNQTALYFCATSEGGPPYEQYFGPGTRLTVTEDLKNVFPPEVAVFEPSEAEISHTQKATLVCLATGFYPDHVELSWWVNGKEVHSGVSTDPQPLKEQPALNDSRYCLSSRLRVSATFWQNPRNHFRCQVQFYGLSENDEWTQDRAKPVTQIVSAEAWGRADCGFTSESYQQGVLSATILYEILLGKATLYAVLVSALVLMAMVKRKDSRG

SEQ ID NO: 15 - protein, 27 aa, Homo sapiens
RAKRSGSGATNFSLLKQAGDVEENPGP

SEQ ID NO: 16 - protein, 6 aa, Homo sapiens
NSAFQY

SEQ ID NO: 17 - protein, 6 aa, Homo sapiens
TYSSGN

SEQ ID NO: 18 - protein, 9 aa, Homo sapiens
AMRGAQKLV

SEQ ID NO: 19 - protein, 5 aa, Homo sapiens
LNHNV

SEQ ID NO: 20 - protein, 6 aa, Homo sapiens
YYDKDF

SEQ ID NO: 21 - protein, 11 aa, Homo sapiens
ATSWDRGYEQY

SEQ ID NO: 22 - protein, 131 aa, Homo sapiens
MMKSLRVLLVILWLQLSWVWSQQKEVEQDPGPLSVPEGAIVSLNCTYSNSAFQYFMWYRQYSRKGPELLMYTYSSGNKEDGRFTAQVDKSSKYISLFIRDSQPSDSATYLCAMRGAQKLVFGQGTRLTINP

SEQ ID NO: 23 - protein, 131 aa, Homo sapiens
MGPGLLHWMALCLLGTGHGDAMVIQNPRYQVTQFGKPVTLSCSQTLNHNVMYWYQQKSSQAPKLLFHYYDKDFNNEADTPDNFQSRRPNTSFCFLDIRSPGLGDAAMYLCATSWDRGYEQYFGPGTRLTVT

SEQ ID NO: 24 - protein, 272 aa, Homo sapiens
MMKSLRVLLVILWLQLSWVWSQQKEVEQDPGPLSVPEGAIVSLNCTYSNSAFQYFMWYRQYSRKGPELLMYTYSSGNKEDGRFTAQVDKSSKYISLFIRDSQPSDSATYLCAMRGAQKLVFGQGTRLTINPNIQNPDPAVYQLRDSKSSDKSVCLFTDFDSQTNVSQSKDSDVYITDKTVLDMRSMDFKSNSAVAWSNKSDFACANAFNNSIIPEDTFFPSPESSCDVKLVEKSFETDTNLNFQNLSVIGFRILLLKVAGFNLLMTLRLWSR

SEQ ID NO: 25 - protein, 310 aa, Homo sapiens
MGPGLLHWMALCLLGTGHGDAMVIQNPRYQVTQFGKPVTLSCSQTLNHNVMYWYQQKSSQAPKLLFHYYDKDFNNEADTPDNFQSRRPNTSFCFLDIRSPGLGDAAMYLCATSWDRGYEQYFGPGTRLTVTEDLKNVFPPEVAVFEPSEAEISHTQKATLVCLATGFYPDHVELSWWVNGKEVHSGVSTDPQPLKEQPALNDSRYCLSSRLRVSATFWQNPRNHFRCQVQFYGLSENDEWTQDRAKPVTQIVSAEAWGRADCGFTSESYQQGVLSATILYEILLGKATLYAVLVSALVLMAMVKRKDSRG

SEQ ID NO: 26 - protein, 6 aa, Homo sapiens
DSASNY

SEQ ID NO: 27 - protein, 7 aa, Homo sapiens
IRSNVGE

SEQ ID NO: 28 - protein, 10 aa, Homo sapiens
AASGATDKLI

SEQ ID NO: 29 - protein, 5 aa, Homo sapiens
MGHDK

SEQ ID NO: 30 - protein, 6 aa, Homo sapiens
SYGVNS

SEQ ID NO: 31 - protein, 9 aa, Homo sapiens
ASSGGHEQY

SEQ ID NO: 32 - protein, 130 aa, Homo sapiens
MTSIRAVFIFLWLQLDLVNGENVEQHPSTLSVQEGDSAVIKCTYSDSASNYFPWYKQELGKRPQLIIDIRSNVGEKKDQRIAVTLNKTAKHFSLHITETQPEDSAVYFCAASGATDKLIFGTGTRLQVFP

SEQ ID NO: 33 - protein, 129 aa, Homo sapiens
MTIRLLCYMGFYFLGAGLMEADIYQTPRYLVIGTGKKITLECSQTMGHDKMYWYQQDPGMELHLIHYSYGVNSTEKGDLSSESTVSRIRTEHFPLTLESARPSHTSQYLCASSGGHEQYFGPGTRLTVT

SEQ ID NO: 34 - protein, 271 aa, Homo sapiens
MTSIRAVFIFLWLQLDLVNGENVEQHPSTLSVQEGDSAVIKCTYSDSASNYFPWYKQELGKRPQLIIDIRSNVGEKKDQRIAVTLNKTAKHFSLHITETQPEDSAVYFCAASGATDKLIFGTGTRLQVFPNIQNPDPAVYQLRDSKSSDKSVCLFTDFDSQTNVSQSKDSDVYITDKTVLDMRSMDFKSNSAVAWSNKSDFACANAFNNSIIPEDTFFPSPESSCDVKLVEKSFETDTNLNFQNLSVIGFRILLLKVAGFNLLMTLRLWSS

SEQ ID NO: 35 - protein, 308 aa, Homo sapiens
MTIRLLCYMGFYFLGAGLMEADIYQTPRYLVIGTGKKITLECSQTMGHDKMYWYQQDPGMELHLIHYSYGVNSTEKGDLSSESTVSRIRTEHFPLTLESARPSHTSQYLCASSGGHEQYFGPGTRLTVTEDLKNVFPPEVAVFEPSEAEISHTQKATLVCLATGFFPDHVELSWWVNGKEVHSGVSTDPQPLKEQPALNDSRYCLSSRLRVSATFWQNPRNHFRCQVQFYGLSENDEWTQDRAKPVTQIVSAEAWGRADCGFTSVSYQQGVLSATILYEILLGKATLYAVLVSALVLMAMVKRKDSRG

SEQ ID NO: 36 - protein, 7 aa, Homo sapiens
TSESDYY

SEQ ID NO: 37 - protein, 8 aa, Homo sapiens
QEAYKQQN

SEQ ID NO: 38 - protein, 13 aa, Homo sapiens
AYRSAQGGSEKLV

SEQ ID NO: 39 - protein, 5 aa, Homo sapiens
LGHNA

SEQ ID NO: 40 - protein, 6 aa, Homo sapiens
YSLEER

SEQ ID NO: 41 - protein, 12 aa, Homo sapiens
ASSQTTYYNEQF

SEQ ID NO: 42 - protein, 137 aa, Homo sapiens
MACPGFLWALVISTCLEFSMAQTVTQSQPEMSVQEAETVTLSCTYDTSESDYYLFWYKQPPSRQMILVIRQEAYKQQNATENRFSVNFQKAAKSFSLKISDSQLGDAAMYFCAYRSAQGGSEKLVFGKGTKLTVNPY

SEQ ID NO: 43 - protein, 132 aa, Homo sapiens
MGCRLLCCAVLCLLGAVPMETGVTQTPRHLVMGMTNKKSLKCEQHLGHNAMYWYKQSAKKPLELMFVYSLEERVENNSVPSRFSPECPNSSHLFLHLHTLQPEDSALYLCASSQTTYYNEQFFGPGTRLTVL

SEQ ID NO: 44 - protein, 277 aa, Homo sapiens
MACPGFLWALVISTCLEFSMAQTVTQSQPEMSVQEAETVTLSCTYDTSESDYYLFWYKQPPSRQMILVIRQEAYKQQNATENRFSVNFQKAAKSFSLKISDSQLGDAAMYFCAYRSAQGGSEKLVFGKGTKLTVNPYIQNPDPAVYQLRDSKSSDKSVCLFTDFDSQTNVSQSKDSDVYITDKTVLDMRSMDFKSNSAVAWSNKSDFACANAFNNSIIPEDTFFPSPESSCDVKLVEKSFETDTNLNFQNLSVIGFRILLLKVAGFNLLMTLRLWSS

SEQ ID NO: 45 - protein, 311 aa, Homo sapiens
MGCRLLCCAVLCLLGAVPMETGVTQTPRHLVMGMTNKKSLKCEQHLGHNAMYWYKQSAKKPLELMFVYSLEERVENNSVPSRFSPECPNSSHLFLHLHTLQPEDSALYLCASSQTTYYNEQFFGPGTRLTVLEDLKNVFPPEVAVFEPSEAEISHTQKATLVCLATGFYPDHVELSWWVNGKEVHSGVSTDPQPLKEQPALNDSRYCLSSRLRVSATFWQNPRNHFRCQVQFYGLSENDEWTQDRAKPVTQIVSAEAWGRADCGFTSESYQQGVLSATILYEILLGKATLYAVLVSALVLMAMVKRKDSRG

SEQ ID NO: 46 - DNA, 1827 bp, Homo sapiens
atgatatccttgagagttttactggtgatcctgtggcttcagttaagctgggtttggagccaacggaaggaggtggagcaggatcctggacccttcaatgttccagagggagccactgtcgctttcaactgtacttacagcaacagtgcttctcagtctttcttctggtacagacaggattgcaggaaagaacctaagttgctgatgtccgtatactccagtggtaatgaagatggaaggtttacagcacagctcaatagagccagccagtatatttccctgctcatcagagactccaagctcagtgattcagccacctacctctgtgtggtgaaccgcgacaatgacatgcgctttggagcagggaccagactgacagtaaaaccaaatatccagaaccctgaccctgccgtgtaccagctgagagactctaaatccagtgacaagtctgtctgcctattcaccgatattgattctcaaacaaatgtgtcacaaagtaaggattctgatgtgtatatcacagacaaaactgtgctagacatgaggtctatggacttcaagagcaacagtgctgtggcctggagcaacaaatctgactttgcatgtgcaaacgccttcaacaacagcattattccagaagacaccttcttccccagcccagaaagttcctgtgatgtcaagctggtcgagaaaagctttgaaacagatacgaacctaaactttcaaaacctgtcagtgattgggttccgaatcctcctcctgaaagtggccgggtttaatctgctcatgacgctgcggctgtggtccagccgggccaagcggtccggatccggagccaccaacttcagcctgctgaagcaggccggcgacgtggaggagaaccccggccccatggcctccctgctcttcttctgtggggccttttatctcctgggaacagggtccatggatgctgatgttacccagaccccaaggaataggatcacaaagacaggaaagaggattatgctggaatgttctcagactaagggtcatgatagaatgtactggtatcgacaagacccaggactgggcctacggttgatctattactcctttgatgtcaaagatataaacaaaggagagatctctgatggatacagtgtctctcgacaggcacaggctaaattctccctgtccctagagtctgccatccccaaccagacagctctttacttctgtgccaccagtgagggagggccgccctacgagcagtacttcgggccgggcaccaggctcacggtcacagaggacctgaaaaacgtgttcccacccgaggtcgctgtgtttgagccatcagaagcagagatctcccacacccaaaaggccacactggtgtgcctggccacaggcttctaccccgaccacgtggagctgagctggtgggtgaatgggaaggaggtgcacagtggggtcagcacagacccgcagcccctcaaggagcagcccgccctcaatgactccagatactgcctgagcagccgcctgagggtctcggccaccttctggcagaacccccgcaaccacttccgctgtcaagtccagttctacgggctctcggagaatgacgagtggacccaggatagggccaaacctgtcacccagatcgtcagcgccgaggcctggggtagagcagactgtggcttcacctccgagtcttaccagcaaggggtcctgtctgccaccatcctctatgagatcttgctagggaaggccaccttgtatgccgtgctggtcagtgccctcgtgctgatggcyatggtcaagagaaaggattccagaggctag

SEQ ID NO: 47 - DNA, 1821 bp, Homo sapiens
atgacatccattcgagctgtatttatattcctgtggctgcagctggacttggtgaatggagagaatgtggagcagcatccttcaaccctgagtgtccaggagggagacagcgctgttatcaagtgtacttattcagacagtgcctcaaactacttcccttggtataagcaagaacttggaaaaagacctcagcttattatagacattcgttcaaatgtgggcgaaaagaaagaccaacgaattgctgttacattgaacaagacagccaaacatttctccctgcacatcacagagacccaacctgaagactcggctgtctacttctgtgcagcaagtggggccaccgacaagctcatctttgggactgggaccagattacaagtctttccaaatatccagaaccctgaccctgccgtgtaccagctgagagactctaaatccagtgacaagtctgtctgcctattcaccgattttgattctcaaacaaatgtgtcacaaagtaaggattctgatgtgtatatcacagacaaaactgtgctagacatgaggtctatggacttcaagagcaacagtgctgtggcctggagcaacaaatctgactttgcatgtgcaaacgccttcaacaacagcattattccagaagacaccttcttccccagcccagaaagttcctgtgatgtcaagctggtcgagaaaagctttgaaacagatacgaacctaaactttcaaaacctgtcagtgattgggttccgaatcctcctcctgaaagtggccgggtttaatctgctcatgacgctgcggctgtggtccagccgggccaagcggtccggatccggagccaccaacttcagcctgctgaagcaggccggcgacgtggaggagaaccccggccccatgactatcaggctcctctgctacatgggcttttattttctgggggcaggcctcatggaagctgacatctaccagaccccaagataccttgttatagggacaggaaagaagatcactctggaatgttctcaaaccatgggccatgacaaaatgtactggtatcaacaagatccaggaatggaactacacctcatccactattcctatggagttaattccacagagaagggagatctttcctccgagtcaacagtctccagaataaggacggagcattttcccctgaccctggagtctgccaggccctcacatacctctcagtacctctgtgccagcagtggcgggcacgagcagtacttcgggccgggcaccaggctcacggtcacagaggacctgaaaaacgtgttcccacccgaggtcgctgtgtttgagccatcagaagcagagatctcccacacccaaaaggccacactggtgtgcctggccacaggcttcttccctgaccacgtggagctgagctggtgggtgaatgggaaggaggtgcacagtggggtcagcacggacccgcagcccctcaaggagcagcccgccctcaatgactccagatactgcctgagcagccgcctgagggtctcggccaccttctggcagaacccccgcaaccacttccgctgtcaagtccagttctacgggctctcggagaatgacgagtggacccaggatagggccaaacccgtcacccagatcgtcagcgccgaggcctggggtagagcagactgtggctttacctcggtgtcctaccagcaaggggtcctgtctgccaccatcctctatgagatcctgctagggaaggccaccctgtatgctgtgctggtcagcgcccttgtgttgatggctatggtcaagagaaaggattccagaggctag

SEQ ID NO: 48 - DNA, 1830 bp, Homo sapiens
atgatgaaatccttgagagttttactggtgatcctgtggcttcagttaagctgggtttggagccaacagaaggaggtggagcaggatcctggaccactcagtgttccagagggagccattgtttctctcaactgcacttacagcaacagtgcttttcaatacttcatgtggtacagacagtattccagaaaaggccctgagttgctgatgtacacatactccagtggtaacaaagaagatggaaggtttacagcacaggtcgataaatccagcaagtatatctccttgttcatcagagactcacagcccagtgattcagccacctacctctgtgcaatgcggggagcccagaagctggtatttggccaaggaaccaggctgactatcaacccaaatatccagaaccctgaccctgccgtgtaccagctgagagactctaaatccagtgacaagtctgtctgcctattcaccgattttgattctcaaacaaatgtgtcacaaagtaaggattctgatgtgtatatcacagacaaaactgtgctagacatgaggtctatggacttcaagagcaacagtgctgtggcctggagcaacaaatctgactttgcatgtgcaaacgccttcaacaacagcattattccagaagacaccttcttccccagcccagaaagttcctgtgatgtcaagctggtcgagaaaagctttgaaacagatacgaacctaaactttcaaaacctgtcagtgattgggttccgaatcctcctcctgaaagtggccgggtttaatctgctcatgacgctgcggctgtggtccagacgggccaagcggtccggatccggagccaccaacttcagcctgctgaagcaggcctgcgacgtggaggagaaccccggccccatgggtcctgggcttctccactggatggccctttgtctccttggaacaggtcatggggatgccatggtcatccagaacccaagataccaggttacccagtttggaaagccagtgaccctgagttgttctcagactttgaaccataacgtcatgtactggtaccagcagaagtcaagtcaggccccaaagctgctgttccactactatgacaaagattttaacaatgaagcagacacccctgataacttccaatccaggaggccgaacacttctttctgctttcttgacatccgctcaccaggcctgggggacgcagccatgtacctgtgtgccacctcctgggaccgagggtacgagcagtacttcgggccgggcaccaggctcacggtcacagaggacctgaaaaacgtgttcccacccgaggtcgctgtgtttgagccatcagaagcagagatctcccacacccaaaaggccacactggtgtgcctggccacaggcttctaccccgaccacgtggagctgagctggtgggtgaatgggaaggaggtgcacagtggggtcagcacagacccgcagcccctcaaggagcagcccgccctcaatgactccagatactgcctgagcagccgcctgagggtctcggccaccttctggcagaacccccgcaaccacttccgctgtcaagtccagttctacgggctctcggagaatgacgagtggacccaggatagggccaaacctgtcacccagatcgtcagcgccgaggcctggggtagagcagactgtggcttcacctccgagtcttaccagcaaggggtcctgtctgccaccatcctctatgagatcttgctagggaaggccaccttgtatgccgtgctggtcagtgccctcgtgctgatggctatggtcaagagaaaggattccagaggctag

SEQ ID NO: 49 - DNA, 1848 bp, Homo sapiens
atggcatgccctggcttcctgtgggcacttgtgatctccacctgtcttgaatttagcatggctcagacagtcactcagtctcaaccagagatgtctgtgcaggaggcagagaccgtgaccctgagctgcacatatgacaccagtgagagtgattattatttattctggtacaagcagcctcccagcaggcagatgattctcgttattcgccaagaagcttataagcaacagaatgcaacagagaatcgtttctctgtgaacttccagaaagcagccaaatccttcagtctcaagatctcagactcacagctgggggatgccgcgatgtatttctgtgcttataggagcgctcagggcggatctgaaaagctggtctttggaaagggaacgaaactgacagtaaacccatatatccagaaccctgaccctgccgtgtaccagctgagagactctaaatccagtgacaagtctgtctgcctattcaccgattttgattctcaaacaaatgtgtcacaaagtaaggattctgatgtgtatatcacagacaaaactgtgctagacatgaggtctatggacttcaagagcaacagtgctgtggcctggagcaacaaatctgactttgcatgtgcaaacgccttcaacaacagcattattccagaagacaccttcttccccagcccagaaagttcctgtgatgtcaagctggtcgagaaaagctttgaaacagatacgaacctaaactttcaaaacctgtcagtgattgggttccgaatcctcctcctgaaagtggccgggtttaatctgctcatgacgctgcggctgtggtccagccgggccaagcggtccggatccggagccaccaacttcagcctgctgaagcaggccggcgacgtggaggagaaccccggccccatgggctgcaggctgctctgctgtgcggttctctgtctcctgggagcggtccccatggaaacgggagttacgcagacaccaagacacctggtcatgggaatgacaaataagaagtctttgaaatgtgaacaacatctgggtcataacgctatgtattggtacaagcaaagtgctaagaagccactggagctcatgtttgtctacagtcttgaagaacgggttgaaaacaacagtgtgccaagtcgcttctcaccggaatgccccaacagctctcacttattccttcacctacacaccctgcagccagaagactcggccctgtatctctgcgccagcagccaaactacttactacaatgagcagttcttcgggccagggacacggctcaccgtgctagaggacctgaaaaacgtgttcccacccgaggtcgctgtgtttgagccatcagaagcagagatctcccacacccaaaaggccacactggtgtgcctggccacaggcttctaccccgaccacgtggagctgagctggtgggtgaatgggaaggaggtgcacagtggggtcagcacagacccgcagcccctcaaggagcagcccgccctcaatgactccagatactgcctgagcagccgcctgagggtctcggccaccttctggcagaacccccgcaaccacttccgctgtcaagtccagttctacgggctctcggagaatgacgagtggacccaggatagggccaaacccgtcacccagatcgtcagcgccgaggcctggggtagagcagactgtggcttcacctccgagtcttaccagcaaggggtcctgtctgccaccatcctctatgagatcttgctagggaaggccaccttgtatgccgtgctggtcagtgccctcgtgctgatggccatggtcaagagaaaggattccagaggctag

SEQ ID NO: 50 - protein, 9 aa, Homo sapiens
VPISHLYIL

SEQ ID NO: 51 - protein, 9 aa, Homo sapiens
DPIGHLYIF

SEQ ID NO: 52 - protein, 9 aa, Homo sapiens
DPIGHVYIF

SEQ ID NO: 53 - protein, 9 aa, Homo sapiens
EDGCPAAEK

SEQ ID NO: 54 - protein, 27 aa, Artificial Sequence
  Synthetic
RAKRSGSGATNFSLLKQACDVEENPGP

SEQ ID NO: 55 - DNA, 20 bp, Artificial Sequence
  Synthetic
cactgttgctcttgaagtcc

SEQ ID NO: 56 - DNA, 24 bp, Artificial Sequence
  Synthetic
caggcagtatctggagtcattgag

SEQ ID NO: 57 - protein, 4 aa, Artificial Sequence
  Synthetic
SGSG

SEQ ID NO: 58 - DNA, 27 bp, Artificial Sequence
  Synthetic
tgcaaggcatggaaaatacataactga

SEQ ID NO: 59 - DNA, 25 bp, Artificial Sequence
  Synthetic
cacagatatcctgtttggcccatat

SEQ ID NO: 60 - DNA, 20 bp, Artificial Sequence
  Synthetic
tctctctgttcctaaccttg

SEQ ID NO: 61 - DNA, 20 bp, Artificial Sequence
  Synthetic
tccgtgaggaggcaaggttc

SEQ ID NO: 62 - DNA, 19 bp, Artificial Sequence
  Synthetic
gagcctgcgcacccaccaa

SEQ ID NO: 63 - DNA, 28 bp, Artificial Sequence
  Synthetic
agtgtgggcaggagctagtgctgctccg